European Patent Specification EP 3 513 806 B1, published January 25, 2023. Title: Immunogenic composition. Applicant: GlaxoSmithKline Biologicals S.A. The sequence listing filed with the application follows.

SEQUENCE LISTING (37 sequences)

SEQ ID NO: 1 - protein, 2710 aa, clostridium difficile
MSLISKEELIKLAYSIRPRENEYKTILTNLDEYNKLTTNNNENKYLQLKKLNESIDVFMNKYKTSSRNRALSNLKKDILKEVILIKNSNTSPVEKNLHFVWIGGEVSDIALEYIKQWADINAEYNIKLWYDSEAFLVNTLKKAIVESSTTEALQLLEEEIQNPQFDNMKFYKKRMEFIYDRQKRFINYYKSQINKPTVPTIDDIIKSHLVSEYNRDETVLESYRTNSLRKINSNHGIDIRANSLFTEQELLNIYSQELLNRGNLAAASDIVRLLALKNFGGVYLDVDMLPGIHSDLFKTISRPSSIGLDRWEMIKLEAIMKYKKYINNYTSENFDKLDQQLKDNFKLIIESKSEKSEIFSKLENLNVSDLEIKIAFALGSVINQALISKQGSYLTNLVIEQVKNRYQFLNQHLNPAIESDNNFTDTTKIFHDSLFNSATAENSMFLTKIAPYLQVGFMPEARSTISLSGPGAYASAYYDFINLQENTIEKTLKASDLIEFKFPENNLSQLTEQEINSLWSFDQASAKYQFEKYVRDYTGGSLSEDNGVDFNKNTALDKNYLLNNKIPSNNVEEAGSKNYVHYIIQLQGDDISYEATCNLFSKNPKNSIIIQRNMNESAKSYFLSDDGESILELNKYRIPERLKNKEKVKVTFIGHGKDEFNTSEFARLSVDSLSNEISSFLDTIKLDISPKNVEVNLLGCNMFSYDFNVEETYPGKLLLSIMDKITSTLPDVNKNSITIGANQYEVRINSEGRKELLAHSGKWINKEEAIMSDLSSKEYIFFDSIDNKLKAKSKNIPGLASISEDIKTLLLDASVSPDTKFILNNLKLNIESSIGDYIYYEKLEPVKNIIHNSIDDLIDEFNLLENVSDELYELKKLNNLDEKYLISFEDISKNNSTYSVRFINKSNGESVYVETEKEIFSKYSEHITKEISTIKNSIITDVNGNLLDNIQLDHTSQVNTLNAAFFIQSLIDYSSNKDVLNDLSTSVKVQLYAQLFSTGLNTIYDSIQLVNLISNAVNDTINVLPTITEGIPIVSTILDGINLGAAIKELLDEHDPLLKKELEAKVGVLAINMSLSIAATVASIVGIGAEVTIFLLPIAGISAGIPSLVNNELILHDKATSVVNYFNHLSESKKYGPLKTEDDKILVPIDDLVISEIDFNNNSIKLGTCNILAMEGGSGHTVTGNIDHFFSSPSISSHIPSLSIYSAIGIETENLDFSKKIMMLPNAPSRVFWWETGAVPGLRSLENDGTRLLDSIRDLYPGKFYWRFYAFFDYAITTLKPVYEDTNIKIKLDKDTRNFIMPTITTNEIRNKLSYSFDGAGGTYSLLLSSYPISTNINLSKDDLWIFNIDNEVREISIENGTIKKGKLIKDVLSKIDINKNKLIIGNQTIDFSGDIDNKDRYIFLTCELDDKISLIIEINLVAKSYSLLLSGDKNYLISNLSNTIEKINTLGLDSKNIAYNYTDESNNKYFGAISKTSQKSIIHYKKDSKNILEFYNDSTLEFNSKDFIAEDINVFMKDDINTITGKYYVDNNTDKSIDFSISLVSKNQVKVNGLYLNESVYSSYLDFVKNSDGHHNTSNFMNLFLDNISFWKLFGFENINFVIDKYFTLVGKTNLGYVEFICDNNKNIDIYFGEWKTSSSKSTIFSGNGRNVVVEPIYNPDTGEDISTSLDFSYEPLYGIDRYINKVLIAPDLYTSLININTNYYSNEYYPEIIVLNPNTFHKKVNINLDSSSFEYKWSTEGSDFILVRYLEESNKKILQKIRIKGILSNTQSFNKMSIDFKDIKKLSLGYIMSNFKSFNSENELDRDHLGFKIIDNKTYYYDEDSKLVKGLININNSLFYFDPIEFNLVTGWQTINGKKYYFDINTGAALTSYKIINGKHFYFNNDGVMQLGVFKGPDGFEYFAPANTQNNNIEGQAIVYQSKFLTLNGKKYYFDNNSKAVTGWRIINNEKYYFNPNNAIAAVGLQVIDNNKYYFNPDTAIISKGWQTVNGSRYYFDTDTAIAFNGYKTIDGKHFYFDSDCVVKIGVFSTSNGFEYFAPANTYNNNIEGQAIVYQSKFLTLNGKKYYFDNNSKAVTGLQTIDSKKYYFNTNTAEAATGWQTIDGKKYYFNTNTAEAATGWQTIDGKKYYFNTNTAIASTGYTIINGKHFYFNTDGIMQIGVFKGPNGFEYFAPANTDANNIEGQAILYQNEFLTLNGKKYYFGSDSKAVTGWRIINNKKYYFNPNNAIAAIHLCTINNDKYYFSYDGILQNGYITIERNNFYFDANNESKMVTGVFKGPNGFEYFAPANTHNNNIEGQAIVYQNKFLTLNGKKYYFDNDSKAVTGWQTIDGKKYYFNLNTAEAATGWQTIDGKKYYFNLNTAEAATGWQTIDGKKYYFNTNTFIASTGYTSINGKHFYFNTDGIMQIGVFKGPNGFEYFAPANTDANNIEGQAILYQNKFLTLNGKKYYFGSDSKAVTGLRTIDGKKYYFNTNTAVAVTGWQTINGKKYYFNTNTSIASTGYTIISGKHFYFNTDGIMQIGVFKGPDGFEYFAPANTDANNIEGQAIRYQNRFLYLHDNIYYFGNNSKAATGWVTIDGNRYYFEPNTAMGANGYKTIDNKNFYFRNGLPQIGVFKGSNGFEYFAPANTDANNIEGQAIRYQNRFLHLLGKIYYFGNNSKAVTGWQTINGKVYYFMPDTAMAAAGGLFEIDGVIYFFGVDGVKAPGIYG

SEQ ID NO: 2 - protein, 2366 aa, Clostridium difficile
MSLVNRKQLEKMANVRFRTQEDEYVAILDALEEYHNMSENTVVEKYLKLKDINSLTDIYIDTYKKSGRNKALKKFKEYLVTEVLELKNNNLTPVEKNLHFVWIGGQINDTAINYINQWKDVNSDYNVNVFYDSNAFLINTLKKTVVESAINDTLESFRENLNDPRFDYNKFFRKRMEIIYDKQKNFINYYKAQREENPELIIDDIVKTYLSNEYSKEIDELNTYIEESLNKITQNSGNDVRNFEEFKNGESFNLYEQELVERWNLAAASDILRISALKEIGGMYLDVDMLPGIQPDLFESIEKPSSVTVDFWEMTKLEAIMKYKEYIPEYTSEHFDMLDEEVQSSFESVLASKSDKSEIFSSLGDMEASPLEVKIAFNSKGIINQGLISVKDSYCSNLIVKQIENRYKILNNSLNPAISEDNDFNTTTNTFIDSIMAEANADNGRFMMELGKYLRVGFFPDVKTTINLSGPEAYAAAYQDLLMFKEGSMNIHLIEADLRNFEISKTNISQSTEQEMASLWSFDDARAKAQFEEYKRNYFEGSLGEDDNLDFSQNIVVDKEYLLEKISSLARSSERGYIHYIVQLQGDKISYEAACNLFAKTPYDSVLFQKNIEDSEIAYYYNPGDGEIQEIDKYKIPSIISDRPKIKLTFIGHGKDEFNTDIFAGFDVDSLSTEIEAAIDLAKEDISPKSIEINLLGCNMFSYSINVEETYPGKLLLKVKDKISELMPSISQDSIIVSANQYEVRINSEGRRELLDHSGEWINKEESIIKDISSKEYISFNPKENKITVKSKNLPELSTLLQEIRNNSNSSDIELEEKVMLTECEINVISNIDTQIVEERIEEAKNLTSDSINYIKDEFKLIESISDALCDLKQQNELEDSHFISFEDISETDEGFSIRFINKETGESIFVETEKTIFSEYANHITEEISKIKGTIFDTVNGKLVKKVNLDTTHEVNTLNAAFFIQSLIEYNSSKESLSNLSVAMKVQVYAQLFSTGLNTITDAAKVVELVSTALDETIDLLPTLSEGLPIIATIIDGVSLGAAIKELSETSDPLLRQEIEAKIGIMAVNLTTATTAIITSSLGIASGFSILLVPLAGISAGIPSLVNNELVLRDKATKVVDYFKHVSLVETEGVFTLLDDKIMMPQDDLVISEIDFNNNSIVLGKCEIWRMEGGSGHTVTDDIDHFFSAPSITYREPHLSIYDVLEVQKEELDLSKDLMVLPNAPNRVFAWETGWTPGLRSLENDGTKLLDRIRDNYEGEFYWRYFAFIADALITTLKPRYEDTNIRINLDSNTRSFIVPIITTEYIREKLSYSFYGSGGTYALSLSQYNMGINIELSESDVWIIDVDNVVRDVTIESDKIKKGDLIEGILSTLSIEENKIILNSHEINFSGEVNGSNGFVSLTFSILEGINAIIEVDLLSKSYKLLISGELKILMLNSNHIQQKIDYIGFNSELQKNIPYSFVDSEGKENGFINGSTKEGLFVSELPDVVLISKVYMDDSKPSFGYYSNNLKDVKVITKDNVNILTGYYLKDDIKISLSLTLQDEKTIKLNSVHLDESGVAEILKFMNRKGNTNTSDSLMSFLESMNIKSIFVNFLQSNIKFILDANFIISGTTSIGQFEFICDENDNIQPYFIKFNTLETNYTLYVGNRQNMIVEPNYDLDDSGDISSTVINFSQKYLYGIDSCVNKVVISPNIYTDEINITPVYETNNTYPEVIVLDANYINEKINVNINDLSIRYVWSNDGNDFILMSTSEENKVSQVKIRFVNVFKDKTLANKLSFNFSDKQDVPVSEIILSFTPSYYEDGLIGYDLGLVSLYNEKFYINNFGMMVSGLIYINDSLYYFKPPVNNLITGFVTVGDDKYYFNPINGGAASIGETIIDDKNYYFNQSGVLQTGVFSTEDGFKYFAPANTLDENLEGEAIDFTGKLIIDENIYYFDDNYRGAVEWKELDGEMHYFSPETGKAFKGLNQIGDYKYYFNSDGVMQKGFVSINDNKHYFDDSGVMKVGYTEIDGKHFYFAENGEMQIGVFNTEDGFKYFAHHNEDLGNEEGEEISYSGILNFNNKIYYFDDSFTAVVGWKDLEDGSKYYFDEDTAEAYIGLSLINDGQYYFNDDGIMQVGFVTINDKVFYFSDSGIIESGVQNIDDNYFYIDDNGIVQIGVFDTSDGYKYFAPANTVNDNIYGQAVEYSGLVRVGEDVYYFGETYTIETGWIYDMENESDKYYFNPETKKACKGINLIDDIKYYFDEKGIMRTGLISFENNNYYFNENGEMQFGYINIEDKMFYFGEDGVMQIGVFNTPDGFKYFAHQNTLDENFEGESINYTGWLDLDEKRYYFTDEYIAATGSVIIDGEEYYFDPDTAQLVISE

SEQ ID NO: 3 - protein, 966 aa, Artificial Sequence
  Fusion 1
MGWQTIDGKKYYFNTNTAIASTGYTIINGKHFYFNTDGIMQIGVFKGPNGFEYFAPANTDANNIEGQAILYQNEFLTLNGKKYYFGSDSKAVTGWRIINNKKYYFNPNNAIAAIHLCTINNDKYYFSYDGILQNGYITIERNNFYFDANNESKMVTGVFKGPNGFEYFAPANTHNNNIEGQAIVYQNKFLTLNGKKYYFDNDSKAVTGWQTIDGKKYYFNLNTAEAATGWQTIDGKKYYFNLNTAEAATGWQTIDGKKYYFNTNTFIASTGYTSINGKHFYFNTDGIMQIGVFKGPNGFEYFAPANTDANNIEGQAILYQNKFLTLNGKKYYFGSDSKAVTGLRTIDGKKYYFNTNTAVAVTGWQTINGKKYYFNTNTSIASTGYTIISGKHFYFNTDGIMQIGVFKGPDGFEYFAPANTDANNIEGQAIRYQNRFLYLHDNIYYFGNNSKAATGWVTIDGNRYYFEPNTAMGANGYKTIDNKNFYFRNGLPQIGVFKGSNGFEYFAPANTDANNIEGQAIRYQNRFLHLLGKIYYFGNNSKAVTGWQTINGKVYYFMPDTAMAAAGGLFEIDGVIYFFGVDGVKAPGFVSINDNKHYFDDSGVMKVGYTEIDGKHFYFAENGEMQIGVFNTEDGFKYFAHHNEDLGNEEGEEISYSGILNFNNKIYYFDDSFTAVVGWKDLEDGSKYYFDEDTAEAYIGLSLINDGQYYFNDDGIMQVGFVTINDKVFYFSDSGIIESGVQNIDDNYFYIDDNGIVQIGVFDTSDGYKYFAPANTVNDNIYGQAVEYSGLVRVGEDVYYFGETYTIETGWIYDMENESDKYYFNPETKKACKGINLIDDIKYYFDEKGIMRTGLISFENNNYYFNENGEMQFGYINIEDKMFYFGEDGVMQIGVFNTPDGFKYFAHQNTLDENFEGESINYTGWLDLDEKRYYFTDEYIAATGSVIIDGEEYYFDPDTAQLVISE

SEQ ID NO: 4 - protein, 966 aa, Artificial Sequence
  Fusion 2
MGWQTIDGKKYYFNTNTAIASTGYTIINGKHFYFNTDGIMQIGVFKGPNGFEYFAPANTDANNIEGQAILYQNEFLTLNGKKYYFGSDSKAVTGWRIINNKKYYFNPNNAIAAIHLCTINNDKYYFSYDGILQNGYITIERNNFYFDANNESKMVTGVFKGPNGFEYFAPANTHNNNIEGQAIVYQNKFLTLNGKKYYFDNDSKAVTGWQTIDGKKYYFNLNTAEAATGWQTIDGKKYYFNLNTAEAATGWQTIDGKKYYFNTNTFIASTGYTSINGKHFYFNTDGIMQIGVFKGPNGFEYFAPANTDANNIEGQAILYQNKFLTLNGKKYYFGSDSKAVTGLRTIDGKKYYFNTNTAVAVTGWQTINGKKYYFNTNTSIASTGYTIISGKHFYFNTDGIMQIGVFKGPDGFEYFAPANTDANNIEGQAIRYQNRFLYLHDNIYYFGNNSKAATGWVTIDGNRYYFEPNTAMGANGYKTIDNKNFYFRNGLPQIGVFKGSNGFEYFAPANTDANNIEGQAIRYQNRFLHLLGKIYYFGNNSKAVTGWQTINGKVYYFMPDTAMAAAGGLNQIGDYKYYFNSDGVMQKGFVSINDNKHYFDDSGVMKVGYTEIDGKHFYFAENGEMQIGVFNTEDGFKYFAHHNEDLGNEEGEEISYSGILNFNNKIYYFDDSFTAVVGWKDLEDGSKYYFDEDTAEAYIGLSLINDGQYYFNDDGIMQVGFVTINDKVFYFSDSGIIESGVQNIDDNYFYIDDNGIVQIGVFDTSDGYKYFAPANTVNDNIYGQAVEYSGLVRVGEDVYYFGETYTIETGWIYDMENESDKYYFNPETKKACKGINLIDDIKYYFDEKGIMRTGLISFENNNYYFNENGEMQFGYINIEDKMFYFGEDGVMQIGVFNTPDGFKYFAHQNTLDENFEGESINYTGWLDLDEKRYYFTDEYIAATGSVIIDGEEYYFDPDTAQLVISE

SEQ ID NO: 5 - protein, 833 aa, Artificial Sequence
  Fusion 3
MGWQTIDGKKYYFNTNTAIASTGYTIINGKHFYFNTDGIMQIGVFKGPNGFEYFAPANTDANNIEGQAILYQNEFLTLNGKKYYFGSDSKAVTGWRIINNKKYYFNPNNAIAAIHLCTINNDKYYFSYDGILQNGYITIERNNFYFDANNESKMVTGVFKGPNGFEYFAPANTHNNNIEGQAIVYQNKFLTLNGKKYYFDNDSKAVTGWQTIDGKKYYFNLNTAEAATGWQTIDGKKYYFNLNTAEAATGWQTIDGKKYYFNTNTFIASTGYTSINGKHFYFNTDGIMQIGVFKGPNGFEYFAPANTDANNIEGQAILYQNKFLTLNGKKYYFGSDSKAVTGLRTIDGKKYYFNTNTAVAVTGWQTINGKKYYFNTNTSIASTGYTIISGKHFYFNTDGIMQIGVFKGPDGFEYFAPANTDANNIEGQAIRYQNRFLYLHDNIYYFGNNSKAATGWVTIDGNRYYFEPNTAMGANGYKTIDNKNFYFRNGLPQIGVFKGSNGFEYFAHHNEDLGNEEGEEISYSGILNFNNKIYYFDDSFTAVVGWKDLEDGSKYYFDEDTAEAYIGLSLINDGQYYFNDDGIMQVGFVTINDKVFYFSDSGIIESGVQNIDDNYFYIDDNGIVQIGVFDTSDGYKYFAPANTVNDNIYGQAVEYSGLVRVGEDVYYFGETYTIETGWIYDMENESDKYYFNPETKKACKGINLIDDIKYYFDEKGIMRTGLISFENNNYYFNENGEMQFGYINIEDKMFYFGEDGVMQIGVFNTPDGFKYFAHQNTLDENFEGESINYTGWLDLDEKRYYFTDEYIAATGSVIIDGEEYYFDPDTAQLVISE

SEQ ID NO: 6 - protein, 1057 aa, Artificial Sequence
  Fusion 4
MGWQTIDGKKYYFNTNTAIASTGYTIINGKHFYFNTDGIMQIGVFKGPNGFEYFAPANTDANNIEGQAILYQNEFLTLNGKKYYFGSDSKAVTGWRIINNKKYYFNPNNAIAAIHLCTINNDKYYFSYDGILQNGYITIERNNFYFDANNESKMVTGVFKGPNGFEYFAPANTHNNNIEGQAIVYQNKFLTLNGKKYYFDNDSKAVTGWQTIDGKKYYFNLNTAEAATGWQTIDGKKYYFNLNTAEAATGWQTIDGKKYYFNTNTFIASTGYTSINGKHFYFNTDGIMQIGVFKGPNGFEYFAPANTDANNIEGQAILYQNKFLTLNGKKYYFGSDSKAVTGLRTIDGKKYYFNTNTAVAVTGWQTINGKKYYFNTNTSIASTGYTIISGKHFYFNTDGIMQIGVFKGPDGFEYFAPANTDANNIEGQAIRYQNRFLYLHDNIYYFGNNSKAATGWVTIDGNRYYFEPNTAMGANGYKTIDNKNFYFRNGLPQIGVFKGSNGFEYFAPANTDANNIEGQAIRYQNRFLHLLGKIYYFGNNSKAVTGWQTINGKVYYFMPDTAMAAAGGETIIDDKNYYFNQSGVLQTGVFSTEDGFKYFAPANTLDENLEGEAIDFTGKLIIDENIYYFDDNYRGAVEWKELDGEMHYFSPETGKAFKGLNQIGDYKYYFNSDGVMQKGFVSINDNKHYFDDSGVMKVGYTEIDGKHFYFAENGEMQIGVFNTEDGFKYFAHHNEDLGNEEGEEISYSGILNFNNKIYYFDDSFTAVVGWKDLEDGSKYYFDEDTAEAYIGLSLINDGQYYFNDDGIMQVGFVTINDKVFYFSDSGIIESGVQNIDDNYFYIDDNGIVQIGVFDTSDGYKYFAPANTVNDNIYGQAVEYSGLVRVGEDVYYFGETYTIETGWIYDMENESDKYYFNPETKKACKGINLIDDIKYYFDEKGIMRTGLISFENNNYYFNENGEMQFGYINIEDKMFYFGEDGVMQIGVFNTPDGFKYFAHQNTLDENFEGESINYTGWLDLDEKRYYFTDEYIAATGSVIIDGEEYYFDPDTAQLVISE

SEQ ID NO: 7 - protein, 971 aa, Artificial Sequence
  Fusion 5
MGWQTIDGKKYYFNTNTAIASTGYTIINGKHFYFNTDGIMQIGVFKGPNGFEYFAPANTDANNIEGQAILYQNEFLTLNGKKYYFGSDSKAVTGWRIINNKKYYFNPNNAIAAIHLCTINNDKYYFSYDGILQNGYITIERNNFYFDANNESKMVTGVFKGPNGFEYFAPANTHNNNIEGQAIVYQNKFLTLNGKKYYFDNDSKAVTGWQTIDGKKYYFNLNTAEAATGWQTIDGKKYYFNLNTAEAATGWQTIDGKKYYFNTNTFIASTGYTSINGKHFYFNTDGIMQIGVFKGPNGFEYFAPANTDANNIEGQAILYQNKFLTLNGKKYYFGSDSKAVTGLRTIDGKKYYFNTNTAVAVTGWQTINGKKYYFNTNTSIASTGYTIISGKHFYFNTDGIMQIGVFKGPDGFEYFAPANTDANNIEGQAIRYQNRFLYLHDNIYYFGNNSKAATGWVTIDGNRYYFEPNTAMGANGYKTIDNKNFYFRNGLPQIGVFKGSNGFEYFAPANTDANNIEGQAIRYQNRFLHLLGKIYYFGNNSKAVTGWQTINGKVYYFMPDTAMAAAGGLFEIDGVIYFFGVDGVKAPGIYGGGFVSINDNKHYFDDSGVMKVGYTEIDGKHFYFAENGEMQIGVFNTEDGFKYFAHHNEDLGNEEGEEISYSGILNFNNKIYYFDDSFTAVVGWKDLEDGSKYYFDEDTAEAYIGLSLINDGQYYFNDDGIMQVGFVTINDKVFYFSDSGIIESGVQNIDDNYFYIDDNGIVQIGVFDTSDGYKYFAPANTVNDNIYGQAVEYSGLVRVGEDVYYFGETYTIETGWIYDMENESDKYYFNPETKKACKGINLIDDIKYYFDEKGIMRTGLISFENNNYYFNENGEMQFGYINIEDKMFYFGEDGVMQIGVFNTPDGFKYFAHQNTLDENFEGESINYTGWLDLDEKRYYFTDEYIAATGSVIIDGEEYYFDPDTAQLVISE

SEQ ID NO: 8 - protein, 321 aa, Artificial Sequence
  individual toxin A fragment
MASTGYTSINGKHFYFNTDGIMQIGVFKGPNGFEYFAPANTDANNIEGQAILYQNKFLTLNGKKYYFGSDSKAVTGLRTIDGKKYYFNTNTAVAVTGWQTINGKKYYFNTNTSIASTGYTIISGKHFYFNTDGIMQIGVFKGPDGFEYFAPANTDANNIEGQAIRYQNRFLYLHDNIYYFGNNSKAATGWVTIDGNRYYFEPNTAMGANGYKTIDNKNFYFRNGLPQIGVFKGSNGFEYFAPANTDANNIEGQAIRYQNRFLHLLGKIYYFGNNSKAVTGWQTINGKVYYFMPDTAMAAAGGLFEIDGVIYFFGVDGVKAP

SEQ ID NO: 9 - protein, 612 aa, Artificial Sequence
  individual toxin B fragment
MILMSTSEENKVSQVKIRFVNVFKDKTLANKLSFNFSDKQDVPVSEIILSFTPSYYEDGLIGYDLGLVSLYNEKFYINNFGMMVSGLIYINDSLYYFKPPVNNLITGFVTVGDDKYYFNPINGGAASIGETIIDDKNYYFNQSGVLQTGVFSTEDGFKYFAPANTLDENLEGEAIDFTGKLIIDENIYYFDDNYRGAVEWKELDGEMHYFSPETGKAFKGLNQIGDYKYYFNSDGVMQKGFVSINDNKHYFDDSGVMKVGYTEIDGKHFYFAENGEMQIGVFNTEDGFKYFAHHNEDLGNEEGEEISYSGILNFNNKIYYFDDSFTAVVGWKDLEDGSKYYFDEDTAEAYIGLSLINDGQYYFNDDGIMQVGFVTINDKVFYFSDSGIIESGVQNIDDNYFYIDDNGIVQIGVFDTSDGYKYFAPANTVNDNIYGQAVEYSGLVRVGEDVYYFGETYTIETGWIYDMENESDKYYFNPETKKACKGINLIDDIKYYFDEKGIMRTGLISFENNNYYFNENGEMQFGYINIEDKMFYFGEDGVMQIGVFNTPDGFKYFAHQNTLDENFEGESINYTGWLDLDEKRYYFTDEYIAATGSVIIDGEEYYFDPDTA

SEQ ID NO: 10 - protein, 587 aa, Artificial Sequence
  toxin A fragment from fusion 1
MGWQTIDGKKYYFNTNTAIASTGYTIINGKHFYFNTDGIMQIGVFKGPNGFEYFAPANTDANNIEGQAILYQNEFLTLNGKKYYFGSDSKAVTGWRIINNKKYYFNPNNAIAAIHLCTINNDKYYFSYDGILQNGYITIERNNFYFDANNESKMVTGVFKGPNGFEYFAPANTHNNNIEGQAIVYQNKFLTLNGKKYYFDNDSKAVTGWQTIDGKKYYFNLNTAEAATGWQTIDGKKYYFNLNTAEAATGWQTIDGKKYYFNTNTFIASTGYTSINGKHFYFNTDGIMQIGVFKGPNGFEYFAPANTDANNIEGQAILYQNKFLTLNGKKYYFGSDSKAVTGLRTIDGKKYYFNTNTAVAVTGWQTINGKKYYFNTNTSIASTGYTIISGKHFYFNTDGIMQIGVFKGPDGFEYFAPANTDANNIEGQAIRYQNRFLYLHDNIYYFGNNSKAATGWVTIDGNRYYFEPNTAMGANGYKTIDNKNFYFRNGLPQIGVFKGSNGFEYFAPANTDANNIEGQAIRYQNRFLHLLGKIYYFGNNSKAVTGWQTINGKVYYFMPDTAMAAAGGLFEIDGVIYFFGVDGVKAP

SEQ ID NO: 11 - protein, 567 aa, Artificial Sequence
  toxin A fragment from fusion 2
MGWQTIDGKKYYFNTNTAIASTGYTIINGKHFYFNTDGIMQIGVFKGPNGFEYFAPANTDANNIEGQAILYQNEFLTLNGKKYYFGSDSKAVTGWRIINNKKYYFNPNNAIAAIHLCTINNDKYYFSYDGILQNGYITIERNNFYFDANNESKMVTGVFKGPNGFEYFAPANTHNNNIEGQAIVYQNKFLTLNGKKYYFDNDSKAVTGWQTIDGKKYYFNLNTAEAATGWQTIDGKKYYFNLNTAEAATGWQTIDGKKYYFNTNTFIASTGYTSINGKHFYFNTDGIMQIGVFKGPNGFEYFAPANTDANNIEGQAILYQNKFLTLNGKKYYFGSDSKAVTGLRTIDGKKYYFNTNTAVAVTGWQTINGKKYYFNTNTSIASTGYTIISGKHFYFNTDGIMQIGVFKGPDGFEYFAPANTDANNIEGQAIRYQNRFLYLHDNIYYFGNNSKAATGWVTIDGNRYYFEPNTAMGANGYKTIDNKNFYFRNGLPQIGVFKGSNGFEYFAPANTDANNIEGQAIRYQNRFLHLLGKIYYFGNNSKAVTGWQTINGKVYYFMPDTAMAAAG

SEQ ID NO: 12 - protein, 505 aa, Artificial Sequence
  toxin A fragment from fusion 3
MGWQTIDGKKYYFNTNTAIASTGYTIINGKHFYFNTDGIMQIGVFKGPNGFEYFAPANTDANNIEGQAILYQNEFLTLNGKKYYFGSDSKAVTGWRIINNKKYYFNPNNAIAAIHLCTINNDKYYFSYDGILQNGYITIERNNFYFDANNESKMVTGVFKGPNGFEYFAPANTHNNNIEGQAIVYQNKFLTLNGKKYYFDNDSKAVTGWQTIDGKKYYFNLNTAEAATGWQTIDGKKYYFNLNTAEAATGWQTIDGKKYYFNTNTFIASTGYTSINGKHFYFNTDGIMQIGVFKGPNGFEYFAPANTDANNIEGQAILYQNKFLTLNGKKYYFGSDSKAVTGLRTIDGKKYYFNTNTAVAVTGWQTINGKKYYFNTNTSIASTGYTIISGKHFYFNTDGIMQIGVFKGPDGFEYFAPANTDANNIEGQAIRYQNRFLYLHDNIYYFGNNSKAATGWVTIDGNRYYFEPNTAMGANGYKTIDNKNFYFRNGLPQIGVFKGSNGFEY

SEQ ID NO: 13 - protein, 567 aa, Artificial Sequence; identical to SEQ ID NO: 11
  toxin A fragment from fusion 4

SEQ ID NO: 14 - protein, 591 aa, Artificial Sequence
  toxin A fragment from fusion 5
MGWQTIDGKKYYFNTNTAIASTGYTIINGKHFYFNTDGIMQIGVFKGPNGFEYFAPANTDANNIEGQAILYQNEFLTLNGKKYYFGSDSKAVTGWRIINNKKYYFNPNNAIAAIHLCTINNDKYYFSYDGILQNGYITIERNNFYFDANNESKMVTGVFKGPNGFEYFAPANTHNNNIEGQAIVYQNKFLTLNGKKYYFDNDSKAVTGWQTIDGKKYYFNLNTAEAATGWQTIDGKKYYFNLNTAEAATGWQTIDGKKYYFNTNTFIASTGYTSINGKHFYFNTDGIMQIGVFKGPNGFEYFAPANTDANNIEGQAILYQNKFLTLNGKKYYFGSDSKAVTGLRTIDGKKYYFNTNTAVAVTGWQTINGKKYYFNTNTSIASTGYTIISGKHFYFNTDGIMQIGVFKGPDGFEYFAPANTDANNIEGQAIRYQNRFLYLHDNIYYFGNNSKAATGWVTIDGNRYYFEPNTAMGANGYKTIDNKNFYFRNGLPQIGVFKGSNGFEYFAPANTDANNIEGQAIRYQNRFLHLLGKIYYFGNNSKAVTGWQTINGKVYYFMPDTAMAAAGGLFEIDGVIYFFGVDGVKAPGIYG

SEQ ID NO: 15 - protein, 379 aa, Artificial Sequence
  toxin B fragment from fusion 1
GFVSINDNKHYFDDSGVMKVGYTEIDGKHFYFAENGEMQIGVFNTEDGFKYFAHHNEDLGNEEGEEISYSGILNFNNKIYYFDDSFTAVVGWKDLEDGSKYYFDEDTAEAYIGLSLINDGQYYFNDDGIMQVGFVTINDKVFYFSDSGIIESGVQNIDDNYFYIDDNGIVQIGVFDTSDGYKYFAPANTVNDNIYGQAVEYSGLVRVGEDVYYFGETYTIETGWIYDMENESDKYYFNPETKKACKGINLIDDIKYYFDEKGIMRTGLISFENNNYYFNENGEMQFGYINIEDKMFYFGEDGVMQIGVFNTPDGFKYFAHQNTLDENFEGESINYTGWLDLDEKRYYFTDEYIAATGSVIIDGEEYYFDPDTAQLVISE

SEQ ID NO: 16 - protein, 399 aa, Artificial Sequence
  toxin B fragment from fusion 2
GLNQIGDYKYYFNSDGVMQKGFVSINDNKHYFDDSGVMKVGYTEIDGKHFYFAENGEMQIGVFNTEDGFKYFAHHNEDLGNEEGEEISYSGILNFNNKIYYFDDSFTAVVGWKDLEDGSKYYFDEDTAEAYIGLSLINDGQYYFNDDGIMQVGFVTINDKVFYFSDSGIIESGVQNIDDNYFYIDDNGIVQIGVFDTSDGYKYFAPANTVNDNIYGQAVEYSGLVRVGEDVYYFGETYTIETGWIYDMENESDKYYFNPETKKACKGINLIDDIKYYFDEKGIMRTGLISFENNNYYFNENGEMQFGYINIEDKMFYFGEDGVMQIGVFNTPDGFKYFAHQNTLDENFEGESINYTGWLDLDEKRYYFTDEYIAATGSVIIDGEEYYFDPDTAQLVISE

SEQ ID NO: 17 - protein, 328 aa, Artificial Sequence
  toxin B fragment from fusion 3
FAHHNEDLGNEEGEEISYSGILNFNNKIYYFDDSFTAVVGWKDLEDGSKYYFDEDTAEAYIGLSLINDGQYYFNDDGIMQVGFVTINDKVFYFSDSGIIESGVQNIDDNYFYIDDNGIVQIGVFDTSDGYKYFAPANTVNDNIYGQAVEYSGLVRVGEDVYYFGETYTIETGWIYDMENESDKYYFNPETKKACKGINLIDDIKYYFDEKGIMRTGLISFENNNYYFNENGEMQFGYINIEDKMFYFGEDGVMQIGVFNTPDGFKYFAHQNTLDENFEGESINYTGWLDLDEKRYYFTDEYIAATGSVIIDGEEYYFDPDTAQLVISE

SEQ ID NO: 18 - protein, 490 aa, Artificial Sequence
  toxin B fragment from fusion 4
GETIIDDKNYYFNQSGVLQTGVFSTEDGFKYFAPANTLDENLEGEAIDFTGKLIIDENIYYFDDNYRGAVEWKELDGEMHYFSPETGKAFKGLNQIGDYKYYFNSDGVMQKGFVSINDNKHYFDDSGVMKVGYTEIDGKHFYFAENGEMQIGVFNTEDGFKYFAHHNEDLGNEEGEEISYSGILNFNNKIYYFDDSFTAVVGWKDLEDGSKYYFDEDTAEAYIGLSLINDGQYYFNDDGIMQVGFVTINDKVFYFSDSGIIESGVQNIDDNYFYIDDNGIVQIGVFDTSDGYKYFAPANTVNDNIYGQAVEYSGLVRVGEDVYYFGETYTIETGWIYDMENESDKYYFNPETKKACKGINLIDDIKYYFDEKGIMRTGLISFENNNYYFNENGEMQFGYINIEDKMFYFGEDGVMQIGVFNTPDGFKYFAHQNTLDENFEGESINYTGWLDLDEKRYYFTDEYIAATGSVIIDGEEYYFDPDTAQLVISE

SEQ ID NO: 19 - protein, 379 aa, Artificial Sequence; identical to SEQ ID NO: 15
  toxin B fragment from fusion 5

SEQ ID NO: 20 - DNA, 3339 bp, Artificial Sequence
  nucleotide sequence of F54 Gly fusion protein
atggcaaccggttggcagaccatcgatggcaaaaaatattattttaataccaacaccgcaattgcaagcaccggctataccattatcaacggcaaacacttttattttaacaccgacggcattatgcagattggtgtgtttaaaggtccgaacggctttgaatactttgcaccggcaaataccgatgccaataatattgaaggccaggccattctgtatcagaatgaatttctgaccctgaacggcaaaaaatactactttggcagcgatagcaaagcagttaccggttggcgcatcatcaacaataagaaatattacttcaacccgaataatgcaattgcagcaattcatctgtgcaccattaacaacgacaaatattatttcagctatgacggtattctgcagaatggctacattaccatcgaacgcaacaacttttatttcgatgccaacaacgaaagcaaaatggtgaccggtgttttcaaaggccctaatggttttgagtatttcgctccggcaaacacccataataacaacattgaaggtcaggcgatcgtttatcagaacaaattcctgacgctgaatggtaagaaatactatttcgataatgacagcaaagccgtgaccggctggcagacaattgacgggaagaaatattactttaatctgaataccgcagaagcagcaaccggttggcaaacgatcgacggtaaaaagtactacttcaacctgaacacagccgaagcagccacaggatggcagactattgatggaaaaaaatactatttcaacaccaacacctttattgcatctaccggttataccagcattaacggtaaacatttctacttcaacaccgatggtatcatgcagatcggcgttttcaaaggtccaaatggtttcgaatactttgcccctgccaatacagatgcaaataacatcgagggtcaggcaatcctgtaccaaaacaaatttctgaccctgaatgggaaaaaatattactttggtagcgattctaaagccgttaccggtctgcgtaccattgatggtaaaaaatactactttaatacgaatacagccgttgcggttacaggctggcagaccattaacgggaaaaaatactattttaacacaaataccagcattgcctcaacgggttataccattatttcgggtaaacacttctactttaataccgatggtattatgcaaatcggagtctttaaaggacctgatgggttcgaatattttgcgcctgcgaacactgatgcgaacaatatcgaaggacaggcaatccgctatcagaatcgctttctgtatctgcacgacaacatctattattttggcaacaattcaaaagcagccaccggctgggttacaattgatggcaaccgctactatttcgaaccgaataccgcaatgggtgcaaatggctacaaaaccatcgataataaaaatttctattttcgcaacggtctgccgcagatcggggtatttaaaggtagcaacggcttcgaatacttcgctccagcgaatacggacgcgaacaatattgagggtcaagcgattcgttatcaaaaccgttttctgcatctgctgggcaaaatctactactttggcaataacagtaaagcagttactggatggcagacaatcaatggtaaagtgtactattttatgccggataccgccatggcagcagccggtggtctgtttgaaattgatggcgtgatctatttttttggtgtggatggtgttaaagcaccgggaatatacggtggtaccggctttgtgaccgtgggtgatgataaatactatttcaatccgattaacggtggtgcagcgagcattggcgaaaccatcatcgatgacaaaaactattatttcaaccagagcggtgtgctgcagaccggtgtgtttagcaccgaagatggctttaaatattttgcgccagcgaacaccctggatgaaaacctggaaggcgaagcgattgattttaccggcaaactgatcatcgatgaaaacatctattacttcgatgataactatcgtggtgcggtggaatggaaagaactggatggcgaaatgcattatttttctccggaaaccggtaaagcgtttaaaggcctgaaccagatcggcgattacaaatactacttcaacagcgatggcgtgatgcagaaaggctttgtgagcatcaacgataacaaacactatttcgatgatagcggtgtgatgaaagtgggctataccgaaattgatggcaaacatttctacttcgcggaaaacggcgaaatgcagattggcgtgttcaataccgaagatggtttcaaatacttcgcgcaccataacgaagatctgggtaacgaagaaggcgaagaaattagctatagcggcatcctgaacttcaacaacaaaatctactactttgatgatagctttaccgcggtggtgggctggaaagatctggaagatggcagcaaatattatttcgatgaagataccgcggaagcgtatattggcctgagcctgattaacgatggccagtactattttaacgatgatggcattatgcaggtgggtttcgtgaccattaatgataaagtgttctatttcagcgatagcggcattattgaaagcggcgtgcagaacattgatgataactacttctacatcgatgataacggcattgtgcagatcggcgtttttgataccagcgatggctacaaatatttcgcaccggccaataccgtgaacgataacatttatggccaggcggtggaatatagcggtctggtgcgtgtgggcgaagatgtgtattatttcggcgaaacctataccatcgaaaccggctggatttatgatatggaaaacgaaagcgataaatattactttaatccggaaacgaaaaaagcgtgcaaaggcattaacctgatcgatgatatcaaatactattttgatgaaaaaggcattatgcgtaccggtctgattagcttcgaaaacaacaactattacttcaacgaaaacggtgaaatgcagttcggctacatcaacatcgaagataaaatgttctacttcggcgaagatggtgttatgcagattggtgtttttaacaccccggatggcttcaaatactttgcccatcagaataccctggatgaaaatttcgaaggtgaaagcattaactataccggctggctggatctggatgaaaaacgctactacttcaccgatgaatacattgcggcgaccggcagcgtgattattgatggcgaagaatactacttcgatccggataccgcgcagctggtgattagcgaacatcatcatcatcaccat

SEQ ID NO: 21 - protein, 1113 aa, Artificial Sequence
  amino acid of F54Gly fusion protein
MATGWQTIDGKKYYFNTNTAIASTGYTIINGKHFYFNTDGIMQIGVFKGPNGFEYFAPANTDANNIEGQAILYQNEFLTLNGKKYYFGSDSKAVTGWRIINNKKYYFNPNNAIAAIHLCTINNDKYYFSYDGILQNGYITIERNNFYFDANNESKMVTGVFKGPNGFEYFAPANTHNNNIEGQAIVYQNKFLTLNGKKYYFDNDSKAVTGWQTIDGKKYYFNLNTAEAATGWQTIDGKKYYFNLNTAEAATGWQTIDGKKYYFNTNTFIASTGYTSINGKHFYFNTDGIMQIGVFKGPNGFEYFAPANTDANNIEGQAILYQNKFLTLNGKKYYFGSDSKAVTGLRTIDGKKYYFNTNTAVAVTGWQTINGKKYYFNTNTSIASTGYTIISGKHFYFNTDGIMQIGVFKGPDGFEYFAPANTDANNIEGQAIRYQNRFLYLHDNIYYFGNNSKAATGWVTIDGNRYYFEPNTAMGANGYKTIDNKNFYFRNGLPQIGVFKGSNGFEYFAPANTDANNIEGQAIRYQNRFLHLLGKIYYFGNNSKAVTGWQTINGKVYYFMPDTAMAAAGGLFEIDGVIYFFGVDGVKAPGIYGGTGFVTVGDDKYYFNPINGGAASIGETIIDDKNYYFNQSGVLQTGVFSTEDGFKYFAPANTLDENLEGEAIDFTGKLIIDENIYYFDDNYRGAVEWKELDGEMHYFSPETGKAFKGLNQIGDYKYYFNSDGVMQKGFVSINDNKHYFDDSGVMKVGYTEIDGKHFYFAENGEMQIGVFNTEDGFKYFAHHNEDLGNEEGEEISYSGILNFNNKIYYFDDSFTAVVGWKDLEDGSKYYFDEDTAEAYIGLSLINDGQYYFNDDGIMQVGFVTINDKVFYFSDSGIIESGVQNIDDNYFYIDDNGIVQIGVFDTSDGYKYFAPANTVNDNIYGQAVEYSGLVRVGEDVYYFGETYTIETGWIYDMENESDKYYFNPETKKACKGINLIDDIKYYFDEKGIMRTGLISFENNNYYFNENGEMQFGYINIEDKMFYFGEDGVMQIGVFNTPDGFKYFAHQNTLDENFEGESINYTGWLDLDEKRYYFTDEYIAATGSVIIDGEEYYFDPDTAQLVISEHHHHHH

SEQ ID NO: 22 - DNA, 3324 bp, Artificial Sequence
  nucleotide sequence of F54 New fusion protein
atggcaaccggttggcagaccatcgatggcaaaaaatattattttaataccaacaccgcaattgcaagcaccggctataccattatcaacggcaaacacttttattttaacaccgacggcattatgcagattggtgtgtttaaaggtccgaacggctttgaatactttgcaccggcaaataccgatgccaataatattgaaggccaggccattctgtatcagaatgaatttctgaccctgaacggcaaaaaatactactttggcagcgatagcaaagcagttaccggttggcgcatcatcaacaataagaaatattacttcaacccgaataatgcaattgcagcaattcatctgtgcaccattaacaacgacaaatattatttcagctatgacggtattctgcagaatggctacattaccatcgaacgcaacaacttttatttcgatgccaacaacgaaagcaaaatggtgaccggtgttttcaaaggccctaatggttttgagtatttcgctccggcaaacacccataataacaacattgaaggtcaggcgatcgtttatcagaacaaattcctgacgctgaatggtaagaaatactatttcgataatgacagcaaagccgtgaccggctggcagacaattgacgggaagaaatattactttaatctgaataccgcagaagcagcaaccggttggcaaacgatcgacggtaaaaagtactacttcaacctgaacacagccgaagcagccacaggatggcagactattgatggaaaaaaatactatttcaacaccaacacctttattgcatctaccggttataccagcattaacggtaaacatttctacttcaacaccgatggtatcatgcagatcggcgttttcaaaggtccaaatggtttcgaatactttgcccctgccaatacagatgcaaataacatcgagggtcaggcaatcctgtaccaaaacaaatttctgaccctgaatgggaaaaaatattactttggtagcgattctaaagccgttaccggtctgcgtaccattgatggtaaaaaatactactttaatacgaatacagccgttgcggttacaggctggcagaccattaacgggaaaaaatactattttaacacaaataccagcattgcctcaacgggttataccattatttcgggtaaacacttctactttaataccgatggtattatgcaaatcggagtctttaaaggacctgatgggttcgaatattttgcgcctgcgaacactgatgcgaacaatatcgaaggacaggcaatccgctatcagaatcgctttctgtatctgcacgacaacatctattattttggcaacaattcaaaagcagccaccggctgggttacaattgatggcaaccgctactatttcgaaccgaataccgcaatgggtgcaaatggctacaaaaccatcgataataaaaatttctattttcgcaacggtctgccgcagatcggggtatttaaaggtagcaacggcttcgaatacttcgctccagcgaatacggacgcgaacaatattgagggtcaagcgattcgttatcaaaaccgttttctgcatctgctgggcaaaatctactactttggcaataacagtaaagcagttactggatggcagacaatcaatggtaaagtgtactattttatgccggataccgccatggcagcagccggtggtctgtttgaaattgatggcgtgatctatttttttggtgtggatggtgttaaagcagttaccggctttgtgaccgtgggtgatgataaatactatttcaatccgattaacggtggtgcagcgagcattggcgaaaccatcatcgatgacaaaaactattatttcaaccagagcggtgtgctgcagaccggtgtgtttagcaccgaagatggctttaaatattttgcgccagcgaacaccctggatgaaaacctggaaggcgaagcgattgattttaccggcaaactgatcatcgatgaaaacatctattacttcgatgataactatcgtggtgcggtggaatggaaagaactggatggcgaaatgcattatttttctccggaaaccggtaaagcgtttaaaggcctgaaccagatcggcgattacaaatactacttcaacagcgatggcgtgatgcagaaaggctttgtgagcatcaacgataacaaacactatttcgatgatagcggtgtgatgaaagtgggctataccgaaattgatggcaaacatttctacttcgcggaaaacggcgaaatgcagattggcgtgttcaataccgaagatggtttcaaatacttcgcgcaccataacgaagatctgggtaacgaagaaggcgaagaaattagctatagcggcatcctgaacttcaacaacaaaatctactactttgatgatagctttaccgcggtggtgggctggaaagatctggaagatggcagcaaatattatttcgatgaagataccgcggaagcgtatattggcctgagcctgattaacgatggccagtactattttaacgatgatggcattatgcaggtgggtttcgtgaccattaatgataaagtgttctatttcagcgatagcggcattattgaaagcggcgtgcagaacattgatgataactacttctacatcgatgataacggcattgtgcagatcggcgtttttgataccagcgatggctacaaatatttcgcaccggccaataccgtgaacgataacatttatggccaggcggtggaatatagcggtctggtgcgtgtgggcgaagatgtgtattatttcggcgaaacctataccatcgaaaccggctggatttatgatatggaaaacgaaagcgataaatattactttaatccggaaacgaaaaaagcgtgcaaaggcattaacctgatcgatgatatcaaatactattttgatgaaaaaggcattatgcgtaccggtctgattagcttcgaaaacaacaactattacttcaacgaaaacggtgaaatgcagttcggctacatcaacatcgaagataaaatgttctacttcggcgaagatggtgttatgcagattggtgtttttaacaccccggatggcttcaaatactttgcccatcagaataccctggatgaaaatttcgaaggtgaaagcattaactataccggctggctggatctggatgaaaaacgctactacttcaccgatgaatacattgcggcgaccggcagcgtgattattgatggcgaagaatactacttcgatccggataccgcgcagctggtgattagcgaacatcatcatcatcaccat

SEQ ID NO: 23 - protein, 1108 aa, Artificial Sequence
  amino acid sequence of F54 New fusion protein
MATGWQTIDGKKYYFNTNTAIASTGYTIINGKHFYFNTDGIMQIGVFKGPNGFEYFAPANTDANNIEGQAILYQNEFLTLNGKKYYFGSDSKAVTGWRIINNKKYYFNPNNAIAAIHLCTINNDKYYFSYDGILQNGYITIERNNFYFDANNESKMVTGVFKGPNGFEYFAPANTHNNNIEGQAIVYQNKFLTLNGKKYYFDNDSKAVTGWQTIDGKKYYFNLNTAEAATGWQTIDGKKYYFNLNTAEAATGWQTIDGKKYYFNTNTFIASTGYTSINGKHFYFNTDGIMQIGVFKGPNGFEYFAPANTDANNIEGQAILYQNKFLTLNGKKYYFGSDSKAVTGLRTIDGKKYYFNTNTAVAVTGWQTINGKKYYFNTNTSIASTGYTIISGKHFYFNTDGIMQIGVFKGPDGFEYFAPANTDANNIEGQAIRYQNRFLYLHDNIYYFGNNSKAATGWVTIDGNRYYFEPNTAMGANGYKTIDNKNFYFRNGLPQIGVFKGSNGFEYFAPANTDANNIEGQAIRYQNRFLHLLGKIYYFGNNSKAVTGWQTINGKVYYFMPDTAMAAAGGLFEIDGVIYFFGVDGVKAVTGFVTVGDDKYYFNPINGGAASIGETIIDDKNYYFNQSGVLQTGVFSTEDGFKYFAPANTLDENLEGEAIDFTGKLIIDENIYYFDDNYRGAVEWKELDGEMHYFSPETGKAFKGLNQIGDYKYYFNSDGVMQKGFVSINDNKHYFDDSGVMKVGYTEIDGKHFYFAENGEMQIGVFNTEDGFKYFAHHNEDLGNEEGEEISYSGILNFNNKIYYFDDSFTAVVGWKDLEDGSKYYFDEDTAEAYIGLSLINDGQYYFNDDGIMQVGFVTINDKVFYFSDSGIIESGVQNIDDNYFYIDDNGIVQIGVFDTSDGYKYFAPANTVNDNIYGQAVEYSGLVRVGEDVYYFGETYTIETGWIYDMENESDKYYFNPETKKACKGINLIDDIKYYFDEKGIMRTGLISFENNNYYFNENGEMQFGYINIEDKMFYFGEDGVMQIGVFNTPDGFKYFAHQNTLDENFEGESINYTGWLDLDEKRYYFTDEYIAATGSVIIDGEEYYFDPDTAQLVISEHHHHHH

SEQ ID NO: 24 - DNA, 3387 bp, Artificial Sequence
  nucleotide sequence of F5 ToxB fusion protein
atggcaaccggttggcagaccatcgatggcaaaaaatattattttaataccaacaccgcaattgcaagcaccggctataccattatcaacggcaaacacttttattttaacaccgacggcattatgcagattggtgtgtttaaaggtccgaacggctttgaatactttgcaccggcaaataccgatgccaataatattgaaggccaggccattctgtatcagaatgaatttctgaccctgaacggcaaaaaatactactttggcagcgatagcaaagcagttaccggttggcgcatcatcaacaataagaaatattacttcaacccgaataatgcaattgcagcaattcatctgtgcaccattaacaacgacaaatattatttcagctatgacggtattctgcagaatggctacattaccatcgaacgcaacaacttttatttcgatgccaacaacgaaagcaaaatggtgaccggtgttttcaaaggccctaatggttttgagtatttcgctccggcaaacacccataataacaacattgaaggtcaggcgatcgtttatcagaacaaattcctgacgctgaatggtaagaaatactatttcgataatgacagcaaagccgtgaccggctggcagacaattgacgggaagaaatattactttaatctgaataccgcagaagcagcaaccggttggcaaacgatcgacggtaaaaagtactacttcaacctgaacacagccgaagcagccacaggatggcagactattgatggaaaaaaatactatttcaacaccaacacctttattgcatctaccggttataccagcattaacggtaaacatttctacttcaacaccgatggtatcatgcagatcggcgttttcaaaggtccaaatggtttcgaatactttgcccctgccaatacagatgcaaataacatcgagggtcaggcaatcctgtaccaaaacaaatttctgaccctgaatgggaaaaaatattactttggtagcgattctaaagccgttaccggtctgcgtaccattgatggtaaaaaatactactttaatacgaatacagccgttgcggttacaggctggcagaccattaacgggaaaaaatactattttaacacaaataccagcattgcctcaacgggttataccattatttcgggtaaacacttctactttaataccgatggtattatgcaaatcggagtctttaaaggacctgatgggttcgaatattttgcgcctgcgaacactgatgcgaacaatatcgaaggacaggcaatccgctatcagaatcgctttctgtatctgcacgacaacatctattattttggcaacaattcaaaagcagccaccggctgggttacaattgatggcaaccgctactatttcgaaccgaataccgcaatgggtgcaaatggctacaaaaccatcgataataaaaatttctattttcgcaacggtctgccgcagatcggggtatttaaaggtagcaacggcttcgaatacttcgctccagcgaatacggacgcgaacaatattgagggtcaagcgattcgttatcaaaaccgttttctgcatctgctgggcaaaatctactactttggcaataacagtaaagcagttactggatggcagacaatcaatggtaaagtgtactattttatgccggataccgccatggcagcagccggtggtctgtttgaaattgatggcgtgatctatttttttggtgtggatggtgttaaagcagtgagcggtctgatttatattaacgatagcctgtattactttaaaccaccggtgaataacctgattaccggctttgtgaccgtgggtgatgataaatactatttcaatccgattaacggtggtgcagcgagcattggcgaaaccatcatcgatgacaaaaactattatttcaaccagagcggtgtgctgcagaccggtgtgtttagcaccgaagatggctttaaatattttgcgccagcgaacaccctggatgaaaacctggaaggcgaagcgattgattttaccggcaaactgatcatcgatgaaaacatctattacttcgatgataactatcgtggtgcggtggaatggaaagaactggatggcgaaatgcattatttttctccggaaaccggtaaagcgtttaaaggcctgaaccagatcggcgattacaaatactacttcaacagcgatggcgtgatgcagaaaggctttgtgagcatcaacgataacaaacactatttcgatgatagcggtgtgatgaaagtgggctataccgaaattgatggcaaacatttctacttcgcggaaaacggcgaaatgcagattggcgtgttcaataccgaagatggtttcaaatacttcgcgcaccataacgaagatctgggtaacgaagaaggcgaagaaattagctatagcggcatcctgaacttcaacaacaaaatctactactttgatgatagctttaccgcggtggtgggctggaaagatctggaagatggcagcaaatattatttcgatgaagataccgcggaagcgtatattggcctgagcctgattaacgatggccagtactattttaacgatgatggcattatgcaggtgggtttcgtgaccattaatgataaagtgttctatttcagcgatagcggcattattgaaagcggcgtgcagaacattgatgataactacttctacatcgatgataacggcattgtgcagatcggcgtttttgataccagcgatggctacaaatatttcgcaccggccaataccgtgaacgataacatttatggccaggcggtggaatatagcggtctggtgcgtgtgggcgaagatgtgtattatttcggcgaaacctataccatcgaaaccggctggatttatgatatggaaaacgaaagcgataaatattactttaatccggaaacgaaaaaagcgtgcaaaggcattaacctgatcgatgatatcaaatactattttgatgaaaaaggcattatgcgtaccggtctgattagcttcgaaaacaacaactattacttcaacgaaaacggtgaaatgcagttcggctacatcaacatcgaagataaaatgttctacttcggcgaagatggtgttatgcagattggtgtttttaacaccccggatggcttcaaatactttgcccatcagaataccctggatgaaaatttcgaaggtgaaagcattaactataccggctggctggatctggatgaaaaacgctactacttcaccgatgaatacattgcggcgaccggcagcgtgattattgatggcgaagaatactacttcgatccggataccgcgcagctggtgattagcgaacatcatcatcatcaccat

SEQ ID NO: 25 - protein, 1129 aa, Artificial Sequence
  amino acid sequence of F5 ToxB fusion protein
MATGWQTIDGKKYYFNTNTAIASTGYTIINGKHFYFNTDGIMQIGVFKGPNGFEYFAPANTDANNIEGQAILYQNEFLTLNGKKYYFGSDSKAVTGWRIINNKKYYFNPNNAIAAIHLCTINNDKYYFSYDGILQNGYITIERNNFYFDANNESKMVTGVFKGPNGFEYFAPANTHNNNIEGQAIVYQNKFLTLNGKKYYFDNDSKAVTGWQTIDGKKYYFNLNTAEAATGWQTIDGKKYYFNLNTAEAATGWQTIDGKKYYFNTNTFIASTGYTSINGKHFYFNTDGIMQIGVFKGPNGFEYFAPANTDANNIEGQAILYQNKFLTLNGKKYYFGSDSKAVTGLRTIDGKKYYFNTNTAVAVTGWQTINGKKYYFNTNTSIASTGYTIISGKHFYFNTDGIMQIGVFKGPDGFEYFAPANTDANNIEGQAIRYQNRFLYLHDNIYYFGNNSKAATGWVTIDGNRYYFEPNTAMGANGYKTIDNKNFYFRNGLPQIGVFKGSNGFEYFAPANTDANNIEGQAIRYQNRFLHLLGKIYYFGNNSKAVTGWQTINGKVYYFMPDTAMAAAGGLFEIDGVIYFFGVDGVKAVSGLIYINDSLYYFKPPVNNLITGFVTVGDDKYYFNPINGGAASIGETIIDDKNYYFNQSGVLQTGVFSTEDGFKYFAPANTLDENLEGEAIDFTGKLIIDENIYYFDDNYRGAVEWKELDGEMHYFSPETGKAFKGLNQIGDYKYYFNSDGVMQKGFVSINDNKHYFDDSGVMKVGYTEIDGKHFYFAENGEMQIGVFNTEDGFKYFAHHNEDLGNEEGEEISYSGILNFNNKIYYFDDSFTAVVGWKDLEDGSKYYFDEDTAEAYIGLSLINDGQYYFNDDGIMQVGFVTINDKVFYFSDSGIIESGVQNIDDNYFYIDDNGIVQIGVFDTSDGYKYFAPANTVNDNIYGQAVEYSGLVRVGEDVYYFGETYTIETGWIYDMENESDKYYFNPETKKACKGINLIDDIKYYFDEKGIMRTGLISFENNNYYFNENGEMQFGYINIEDKMFYFGEDGVMQIGVFNTPDGFKYFAHQNTLDENFEGESINYTGWLDLDEKRYYFTDEYIAATGSVIIDGEEYYFDPDTAQLVISEHHHHHH

SEQ ID NO: 26 - DNA, 2985 bp, Artificial Sequence
  nucleotide sequence of F52 new fusion protein
atggcaaccggttggcagaccatcgatggcaaaaaatattattttaataccaacaccgcaattgcaagcaccggctataccattatcaacggcaaacacttttattttaacaccgacggcattatgcagattggtgtgtttaaaggtccgaacggctttgaatactttgcaccggcaaataccgatgccaataatattgaaggccaggccattctgtatcagaatgaatttctgaccctgaacggcaaaaaatactactttggcagcgatagcaaagcagttaccggttggcgcatcatcaacaataagaaatattacttcaacccgaataatgcaattgcagcaattcatctgtgcaccattaacaacgacaaatattatttcagctatgacggtattctgcagaatggctacattaccatcgaacgcaacaacttttatttcgatgccaacaacgaaagcaaaatggtgaccggtgttttcaaaggccctaatggttttgagtatttcgctccggcaaacacccataataacaacattgaaggtcaggcgatcgtttatcagaacaaattcctgacgctgaatggtaagaaatactatttcgataatgacagcaaagccgtgaccggctggcagacaattgacgggaagaaatattactttaatctgaataccgcagaagcagcaaccggttggcaaacgatcgacggtaaaaagtactacttcaacctgaacacagccgaagcagccacaggatggcagactattgatggaaaaaaatactatttcaacaccaacacctttattgcatctaccggttataccagcattaacggtaaacatttctacttcaacaccgatggtatcatgcagatcggcgttttcaaaggtccaaatggtttcgaatactttgcccctgccaatacagatgcaaataacatcgagggtcaggcaatcctgtaccaaaacaaatttctgaccctgaatgggaaaaaatattactttggtagcgattctaaagccgttaccggtctgcgtaccattgatggtaaaaaatactactttaatacgaatacagccgttgcggttacaggctggcagaccattaacgggaaaaaatactattttaacacaaataccagcattgcctcaacgggttataccattatttcgggtaaacacttctactttaataccgatggtattatgcaaatcggagtctttaaaggacctgatgggttcgaatattttgcgcctgcgaacactgatgcgaacaatatcgaaggacaggcaatccgctatcagaatcgctttctgtatctgcacgacaacatctattattttggcaacaattcaaaagcagccaccggctgggttacaattgatggcaaccgctactatttcgaaccgaataccgcaatgggtgcaaatggctacaaaaccatcgataataaaaatttctattttcgcaacggtctgccgcagatcggggtatttaaaggtagcaacggcttcgaatacttcgctccagcgaatacggacgcgaacaatattgagggtcaagcgattcgttatcaaaaccgttttctgcatctgctgggcaaaatctactactttggcaataacagtaaagcagttactggatggcagacaatcaatggtaaagtgtactattttatgccggataccgccatggcagcagccggtggtctgtttgaaattgatggcgtgatctatttttttggtgtggatggtgttaaagcagtgaaaggcctgaaccagatcggcgattacaaatactacttcaacagcgatggcgtgatgcagaaaggctttgtgagcatcaacgataacaaacactatttcgatgatagcggtgtgatgaaagtgggctataccgaaattgatggcaaacatttctacttcgcggaaaacggcgaaatgcagattggcgtgttcaataccgaagatggtttcaaatacttcgcgcaccataacgaagatctgggtaacgaagaaggcgaagaaattagctatagcggcatcctgaacttcaacaacaaaatctactactttgatgatagctttaccgcggtggtgggctggaaagatctggaagatggcagcaaatattatttcgatgaagataccgcggaagcgtatattggcctgagcctgattaacgatggccagtactattttaacgatgatggcattatgcaggtgggtttcgtgaccattaatgataaagtgttctatttcagcgatagcggcattattgaaagcggcgtgcagaacattgatgataactacttctacatcgatgataacggcattgtgcagatcggcgtttttgataccagcgatggctacaaatatttcgcaccggccaataccgtgaacgataacatttatggccaggcggtggaatatagcggtctggtgcgtgtgggcgaagatgtgtattatttcggcgaaacctataccatcgaaaccggctggatttatgatatggaaaacgaaagcgataaatattactttaatccggaaacgaaaaaagcgtgcaaaggcattaacctgatcgatgatatcaaatactattttgatgaaaaaggcattatgcgtaccggtctgattagcttcgaaaacaacaactattacttcaacgaaaacggtgaaatgcagttcggctacatcaacatcgaagataaaatgttctacttcggcgaagatggtgttatgcagattggtgtttttaacaccccggatggcttcaaatactttgcccatcagaataccctggatgaaaatttcgaaggtgaaagcattaactataccggctggctggatctggatgaaaaacgctactacttcaccgatgaatacattgcggcgaccggcagcgtgattattgatggcgaagaatactacttcgatccggataccgcgcagctggtgattagcgaacatcatcatcatcaccat

SEQ ID NO: 27 - protein, 995 aa, Artificial Sequence
  amino acid sequence of F52 New fusion protein
MATGWQTIDGKKYYFNTNTAIASTGYTIINGKHFYFNTDGIMQIGVFKGPNGFEYFAPANTDANNIEGQAILYQNEFLTLNGKKYYFGSDSKAVTGWRIINNKKYYFNPNNAIAAIHLCTINNDKYYFSYDGILQNGYITIERNNFYFDANNESKMVTGVFKGPNGFEYFAPANTHNNNIEGQAIVYQNKFLTLNGKKYYFDNDSKAVTGWQTIDGKKYYFNLNTAEAATGWQTIDGKKYYFNLNTAEAATGWQTIDGKKYYFNTNTFIASTGYTSINGKHFYFNTDGIMQIGVFKGPNGFEYFAPANTDANNIEGQAILYQNKFLTLNGKKYYFGSDSKAVTGLRTIDGKKYYFNTNTAVAVTGWQTINGKKYYFNTNTSIASTGYTIISGKHFYFNTDGIMQIGVFKGPDGFEYFAPANTDANNIEGQAIRYQNRFLYLHDNIYYFGNNSKAATGWVTIDGNRYYFEPNTAMGANGYKTIDNKNFYFRNGLPQIGVFKGSNGFEYFAPANTDANNIEGQAIRYQNRFLHLLGKIYYFGNNSKAVTGWQTINGKVYYFMPDTAMAAAGGLFEIDGVIYFFGVDGVKAVKGLNQIGDYKYYFNSDGVMQKGFVSINDNKHYFDDSGVMKVGYTEIDGKHFYFAENGEMQIGVFNTEDGFKYFAHHNEDLGNEEGEEISYSGILNFNNKIYYFDDSFTAVVGWKDLEDGSKYYFDEDTAEAYIGLSLINDGQYYFNDDGIMQVGFVTINDKVFYFSDSGIIESGVQNIDDNYFYIDDNGIVQIGVFDTSDGYKYFAPANTVNDNIYGQAVEYSGLVRVGEDVYYFGETYTIETGWIYDMENESDKYYFNPETKKACKGINLIDDIKYYFDEKGIMRTGLISFENNNYYFNENGEMQFGYINIEDKMFYFGEDGVMQIGVFNTPDGFKYFAHQNTLDENFEGESINYTGWLDLDEKRYYFTDEYIAATGSVIIDGEEYYFDPDTAQLVISEHHHHHH

SEQ ID NO: 28 - protein, 593 aa, Artificial Sequence
  toxin A fragment of F54 Gly
MATGWQTIDGKKYYFNTNTAIASTGYTIINGKHFYFNTDGIMQIGVFKGPNGFEYFAPANTDANNIEGQAILYQNEFLTLNGKKYYFGSDSKAVTGWRIINNKKYYFNPNNAIAAIHLCTINNDKYYFSYDGILQNGYITIERNNFYFDANNESKMVTGVFKGPNGFEYFAPANTHNNNIEGQAIVYQNKFLTLNGKKYYFDNDSKAVTGWQTIDGKKYYFNLNTAEAATGWQTIDGKKYYFNLNTAEAATGWQTIDGKKYYFNTNTFIASTGYTSINGKHFYFNTDGIMQIGVFKGPNGFEYFAPANTDANNIEGQAILYQNKFLTLNGKKYYFGSDSKAVTGLRTIDGKKYYFNTNTAVAVTGWQTINGKKYYFNTNTSIASTGYTIISGKHFYFNTDGIMQIGVFKGPDGFEYFAPANTDANNIEGQAIRYQNRFLYLHDNIYYFGNNSKAATGWVTIDGNRYYFEPNTAMGANGYKTIDNKNFYFRNGLPQIGVFKGSNGFEYFAPANTDANNIEGQAIRYQNRFLHLLGKIYYFGNNSKAVTGWQTINGKVYYFMPDTAMAAAGGLFEIDGVIYFFGVDGVKAPGIYG

SEQ ID NO: 29 - protein, 589 aa, Artificial Sequence
  toxin A fragment of F54 New
MATGWQTIDGKKYYFNTNTAIASTGYTIINGKHFYFNTDGIMQIGVFKGPNGFEYFAPANTDANNIEGQAILYQNEFLTLNGKKYYFGSDSKAVTGWRIINNKKYYFNPNNAIAAIHLCTINNDKYYFSYDGILQNGYITIERNNFYFDANNESKMVTGVFKGPNGFEYFAPANTHNNNIEGQAIVYQNKFLTLNGKKYYFDNDSKAVTGWQTIDGKKYYFNLNTAEAATGWQTIDGKKYYFNLNTAEAATGWQTIDGKKYYFNTNTFIASTGYTSINGKHFYFNTDGIMQIGVFKGPNGFEYFAPANTDANNIEGQAILYQNKFLTLNGKKYYFGSDSKAVTGLRTIDGKKYYFNTNTAVAVTGWQTINGKKYYFNTNTSIASTGYTIISGKHFYFNTDGIMQIGVFKGPDGFEYFAPANTDANNIEGQAIRYQNRFLYLHDNIYYFGNNSKAATGWVTIDGNRYYFEPNTAMGANGYKTIDNKNFYFRNGLPQIGVFKGSNGFEYFAPANTDANNIEGQAIRYQNRFLHLLGKIYYFGNNSKAVTGWQTINGKVYYFMPDTAMAAAGGLFEIDGVIYFFGVDGVKAV

SEQ ID NO: 30 - protein, 589 aa, Artificial Sequence; identical to SEQ ID NO: 29
  toxin A fragment of F5 ToxB

SEQ ID NO: 31 - protein, 589 aa, Artificial Sequence; identical to SEQ ID NO: 29
  toxin A fragment of F52 New

SEQ ID NO: 32 - protein, 513 aa, Artificial Sequence
  toxin B fragment of F54Gly
TGFVTVGDDKYYFNPINGGAASIGETIIDDKNYYFNQSGVLQTGVFSTEDGFKYFAPANTLDENLEGEAIDFTGKLIIDENIYYFDDNYRGAVEWKELDGEMHYFSPETGKAFKGLNQIGDYKYYFNSDGVMQKGFVSINDNKHYFDDSGVMKVGYTEIDGKHFYFAENGEMQIGVFNTEDGFKYFAHHNEDLGNEEGEEISYSGILNFNNKIYYFDDSFTAVVGWKDLEDGSKYYFDEDTAEAYIGLSLINDGQYYFNDDGIMQVGFVTINDKVFYFSDSGIIESGVQNIDDNYFYIDDNGIVQIGVFDTSDGYKYFAPANTVNDNIYGQAVEYSGLVRVGEDVYYFGETYTIETGWIYDMENESDKYYFNPETKKACKGINLIDDIKYYFDEKGIMRTGLISFENNNYYFNENGEMQFGYINIEDKMFYFGEDGVMQIGVFNTPDGFKYFAHQNTLDENFEGESINYTGWLDLDEKRYYFTDEYIAATGSVIIDGEEYYFDPDTAQLVISE

SEQ ID NO: 33 - protein, 513 aa, Artificial Sequence; identical to SEQ ID NO: 32
  toxin B fragment of F54 New

SEQ ID NO: 34 - protein, 534 aa, Artificial Sequence
  toxin B fragment of F5 ToxB
SGLIYINDSLYYFKPPVNNLITGFVTVGDDKYYFNPINGGAASIGETIIDDKNYYFNQSGVLQTGVFSTEDGFKYFAPANTLDENLEGEAIDFTGKLIIDENIYYFDDNYRGAVEWKELDGEMHYFSPETGKAFKGLNQIGDYKYYFNSDGVMQKGFVSINDNKHYFDDSGVMKVGYTEIDGKHFYFAENGEMQIGVFNTEDGFKYFAHHNEDLGNEEGEEISYSGILNFNNKIYYFDDSFTAVVGWKDLEDGSKYYFDEDTAEAYIGLSLINDGQYYFNDDGIMQVGFVTINDKVFYFSDSGIIESGVQNIDDNYFYIDDNGIVQIGVFDTSDGYKYFAPANTVNDNIYGQAVEYSGLVRVGEDVYYFGETYTIETGWIYDMENESDKYYFNPETKKACKGINLIDDIKYYFDEKGIMRTGLISFENNNYYFNENGEMQFGYINIEDKMFYFGEDGVMQIGVFNTPDGFKYFAHQNTLDENFEGESINYTGWLDLDEKRYYFTDEYIAATGSVIIDGEEYYFDPDTAQLVISE

SEQ ID NO: 35 - protein, 400 aa, Artificial Sequence
  toxin B fragment of F52 New
KGLNQIGDYKYYFNSDGVMQKGFVSINDNKHYFDDSGVMKVGYTEIDGKHFYFAENGEMQIGVFNTEDGFKYFAHHNEDLGNEEGEEISYSGILNFNNKIYYFDDSFTAVVGWKDLEDGSKYYFDEDTAEAYIGLSLINDGQYYFNDDGIMQVGFVTINDKVFYFSDSGIIESGVQNIDDNYFYIDDNGIVQIGVFDTSDGYKYFAPANTVNDNIYGQAVEYSGLVRVGEDVYYFGETYTIETGWIYDMENESDKYYFNPETKKACKGINLIDDIKYYFDEKGIMRTGLISFENNNYYFNENGEMQFGYINIEDKMFYFGEDGVMQIGVFNTPDGFKYFAHQNTLDENFEGESINYTGWLDLDEKRYYFTDEYIAATGSVIIDGEEYYFDPDTAQLVISE

SEQ ID NO: 36 - protein, 958 aa, Artificial Sequence
  C-TAB.G5 fusion
MVTGVFKGPNGFEYFAPANTHNNNIEGQAIVYQNKFLTLNGKKYYFDNDSKAVTGWQTIDGKKYYFNLNTAEAATGWQTIDGKKYYFNLNTAEAATGWQTIDGKKYYFNTNTFIASTGYTSINGKHFYFNTDGIMQIGVFKGPNGFEYFAPANTHNNNIEGQAILYQNKFLTLNGKKYYFGSDSKAVTGLRTIDGKKYYFNTNTAVAVTGWQTINGKKYYFNTNTSIASTGYTIISGKHFYFNTDGIMQIGVFKGPDGFEYFAPANTDANNIEGQAIRYQNRFLYLHDNIYYFGNNSKAATGWVTIDGNRYYFEPNTAMGANGYKTIDNKNFYFRNGLPQIGVFKGSNGFEYFAPANTDANNIEGQAIRYQNRFLHLLGKIYYFGNNSKAVTGWQTINGKVYYFMPDTAMAAAGGLFEIDGVIYFFGVDGVKAPGIYGRSMHNLITGFVTVGDDKYYFNPINGGAASIGETIIDDKNYYFNQSGVLQTGVFSTEDGFKYFAPANTLDENLEGEAIDFTGKLIIDENIYYFDDNYRGAVEWKELDGEMHYFSPETGKAFKGLNQIGDYKYYFNSDGVMQKGFVSINDNKHYFDDSGVMKVGYTEIDGKHFYFAENGEMQIGVFNTEDGFKYFAHHNEDLGNEEGEEISYSGILNFNNKIYYFDDSFTAVVGWKDLEDGSKYYFDEDTAEAYIGLSLINDGQYYFNDDGIMQVGFVTINDKVFYFSDSGIIESGVQNIDDNYFYIDDNGIVQIGVFDTSDGYKYFAPANTVNDNIYGQAVEYSGLVRVGEDVYYFGETYTIETGWIYDMENESDKYYFNPETKKACKGINLIDDIKYYFDEKGIMRTGLISFENNNYYFNENGEMQFGYINIEDKMFYFGEDGVMQIGVFNTPDGFKYFAHQNTLDENFEGESINYTGWLDLDEKRYYFTDEYIAATGSVIIDGEEYYFDPDTAQLVISE

SEQ ID NO: 37 - protein, 957 aa, Artificial Sequence
  C-TAB.G5.1 fusion
VTGVFKGPNGFEYFAPANTHNNNIEGQAIVYQNKFLTLNGKKYYFDNDSKAVTGWQTIDGKKYYFNLNTAEAATGWQTIDGKKYYFNLNTAEAATGWQTIDGKKYYFNTNTFIASTGYTSINGKHFYFNTDGIMQIGVFKGPNGFEYFAPANTDANNIEGQAILYQNKFLTLNGKKYYFGSDSKAVTGLRTIDGKKYYFNTNTAVAVTGWQTINGKKYYFNTNTSIASTGYTIISGKHFYFNTDGIMQIGVFKGPDGFEYFAPANTDANNIEGQAIRYQNRFLYLHDNIYYFGNNSKAATGWVTIDGNRYYFEPNTAMGANGYKTIDNKNFYFRNGLPQIGVFKGSNGFEYFAPANTDANNIEGQAIRYQNRFLHLLGKIYYFGNNSKAVTGWQTINGKVYYFMPDTAMAAAGGLFEIDGVIYFFGVDGVKAPGIYGRSMHNLITGFVTVGDDKYYFNPINGGAASIGETIIDDKNYYFNQSGVLQTGVFSTEDGFKYFAPANTLDENLEGEAIDFTGKLIIDENIYYFDDNYRGAVEWKELDGEMHYFSPETGKAFKGLNQIGDYKYYFNSDGVMQKGFVSINDNKHYFDDSGVMKVGYTEIDGKHFYFAENGEMQIGVFNTEDGFKYFAHHNEDLGNEEGEEISYSGILNFNNKIYYFDDSFTAVVGWKDLEDGSKYYFDEDTAEAYIGLSLINDGQYYFNDDGIMQVGFVTINDKVFYFSDSGIIESGVQNIDDNYFYIDDNGIVQIGVFDTSDGYKYFAPANTVNDNIYGQAVEYSGLVRVGEDVYYFGETYTIETGWIYDMENESDKYYFNPETKKACKGINLIDDIKYYFDEKGIMRTGLISFENNNYYFNENGEMQFGYINIEDKMFYFGEDGVMQIGVFNTPDGFKYFAHQNTLDENFEGESINYTGWLDLDEKRYYFTDEYIAATGSVIIDGEEYYFDPDTAQLVISE